European Patent Specification EP 4 281 584 B1, published April 8, 2026. Title: Target-dependent polymerisation of oligonucleotides. Applicant: Qbiotix Limited. The sequence listing filed with the application follows.

SEQUENCE LISTING (25 sequences)

SEQ ID NO: 1 - DNA, 78 bp, Artificial
  Synthetic
attcagtgcatccttacataataaatcatctggtaatttataattataatcagcaatttatgtaaggatgcactgaat

SEQ ID NO: 2 - DNA, 71 bp, Artificial
  Synthetic
attcagtgcatccttacataatctgacttcatcacctctaattacaaatgttatgtaaggatgcactgaat

SEQ ID NO: 3 - DNA, 44 bp, Artificial
  Synthetic
atggtcatgtgtggcggttcactatatgttaaaccaggtggaac

SEQ ID NO: 4 - DNA, 21 bp, Artificial
  Synthetic
ttatgtaaggatgcactgaat

SEQ ID NO: 5 - DNA, 66 bp, Artificial
  Synthetic
ttacattgtttaccatgcttttgaattcatctaggattctaattaaaagcatggtaaacaatgtaa

SEQ ID NO: 6 - DNA, 66 bp, Artificial
  Synthetic
taacttgatccatgattcattaaaaagcatggtaaacaatgtaataatgaatcatggatcaagtta

SEQ ID NO: 7 - DNA, 66 bp, Artificial
  Synthetic
ttactaaggattagtaccagtataatgaatcatggatcaagttatactggtactaatccttagtaa

SEQ ID NO: 8 - DNA, 66 bp, Artificial
  Synthetic
tcatactagactacctgctatatactggtactaatccttagtaatatagcaggtagtctagtatga

SEQ ID NO: 9 - DNA, 74 bp, Artificial
  Synthetic
ttacattgtttaccatgctttttatagcaggtagtctagtatgaaaaagcatggtaaacaatgtaagccggccc

SEQ ID NO: 10 - DNA, 61 bp, Artificial
  Synthetic
ttacattgtttaccatgcttttgggccggcttacattgtttaccaatggtaaacaatgtaa

SEQ ID NO: 11 - DNA, 22 bp, Artificial
  Synthetic
attatgtaaggatgcactgaat

SEQ ID NO: 12 - DNA, 71 bp, Artificial
  Synthetic
attcagtgcatccttacataatgactgaagtagtggagattaatgtttacttatgtaaggatgcactgaat

SEQ ID NO: 13 - DNA, 78 bp, Artificial
  Synthetic
attcagtgcatccttacataattttagtagaccattaaatattaatattagtcgttattatgtaaggatgcactgaat

SEQ ID NO: 14 - DNA, 28 bp, Artificial
  Synthetic
atgtgagattaaagttaactacatctac

SEQ ID NO: 15 - DNA, 54 bp, Artificial
  Synthetic
ttacacactcagacctagctaaattcagtgcatccttacataatttagctaggt

SEQ ID NO: 16 - DNA, 57 bp, Artificial
  Synthetic
taacttgatccatgattcattattagctaggtctgagtgtgtaataatgaatcatgg

SEQ ID NO: 17 - DNA, 58 bp, Artificial
  Synthetic
ttactaaggattagtaccagtataatgaatcatggatcaagttatactggtactaatc

SEQ ID NO: 18 - DNA, 54 bp, Artificial
  Synthetic
tcatcctagcctaccggctatatactggtactaatccttagtaatatagccggt

SEQ ID NO: 19 - DNA, 66 bp, Artificial
  Synthetic
ttacacactcagacctagctaatatagccggtaggctaggatgattagctaggtctgagtgtgtaa

SEQ ID NO: 20 - DNA, 54 bp, Artificial
  Synthetic
ttacacactcagacctagctaattacacactcagacctagctaattagctaggt

SEQ ID NO: 21 - DNA, 53 bp, Artificial
  Synthetic
accactgtctacctaccttcagtgcatccttacataggtaggtagacagtggt

SEQ ID NO: 22 - DNA, 58 bp, Artificial
  Synthetic
tttcttgatccatgattctttagggtaggtagacagattagaatcatggatcaagaaa

SEQ ID NO: 23 - DNA, 55 bp, Artificial
  Synthetic
aagttcataactatggatcaagaatcatggatcaatgatccatagttatgaactt

SEQ ID NO: 24 - DNA, 60 bp, Artificial
  Synthetic
accactgtctacctaccgatccatagttatgaacggtaggtagacagtggtattagtggc

SEQ ID NO: 25 - DNA, 65 bp, Artificial
  Synthetic
accactgtctacctaccagaagccactaataccactgtctaccagagggtaggtagacagtggta